European Patent Application EP 4 328 327 A2, published February 28, 2024. Title: Reporter Dye For Isothermal Nucleic Acid Amplification, Isothermal-Based Dual Functional Oligonucleotide Containing Quencher, and Method For Nucleic Acid Amplification and Measurement Using Same. Applicant: SD biosensor, Inc. The sequence listing filed with the application follows.

SEQUENCE LISTING (23 sequences)

SEQ ID NO: 1 - DNA, 20 bp, synthetic construct
  misc_feature 1..20: note = Oligonucleotide
  source 1..20: mol_type = other DNA
gtgtgttcaagtacagcatt

SEQ ID NO: 2 - DNA, 20 bp, synthetic construct
  misc_feature 1..20: note = Oligonucleotide
  source 1..20: mol_type = other DNA
ataagggaggatgatcaagg

SEQ ID NO: 3 - DNA, 47 bp, synthetic construct
  misc_feature 1..47: note = Oligonucleotide
  source 1..47: mol_type = other DNA
acctggtgttagatgtttatctgaggccaaacattattttgatagcc

SEQ ID NO: 4 - DNA, 50 bp, synthetic construct
  misc_feature 1..50: note = Oligonucleotide
  source 1..50: mol_type = other DNA
tacattaagaggaaccaatttccgctgatagaattcccacaataagtctt

SEQ ID NO: 5 - DNA, 47 bp, synthetic construct
  misc_feature 1..47: note = Oligonucleotide
  variation 7: note = mutation - n= Amino-C6(or C2)-deoxythymine
  variation 40: note = mutation - n= Amino-C6(or C2)-deoxythymine
  source 1..47: mol_type = other DNA
acctggngttagatgtttatctgaggccaaacattatttngatagcc

SEQ ID NO: 6 - DNA, 47 bp, synthetic construct
  misc_feature 1..47: note = Oligonucleotide
  variation 10: note = mutation - n=Amino-C6(or C2)-deoxythymine
  variation 35: note = mutation - n=Amino-C6(or C2)-deoxythymine
  source 1..47: mol_type = other DNA
acctggtgtnagatgtttatctgaggccaaacatnattttgatagcc

SEQ ID NO: 7 - DNA, 47 bp, synthetic construct
  misc_feature 1..47: note = Oligonucleotide
  variation 14: note = mutation - n=Amino-C6(or C2)-deoxythymine
  variation 35: note = mutation - n=Amino-C6(or C2)-deoxythymine
  source 1..47: mol_type = other DNA
acctggtgttagangtttatctgaggccaaacatnattttgatagcc

SEQ ID NO: 8 - DNA, 50 bp, synthetic construct
  misc_feature 1..50: note = Oligonucleotide
  variation 5: note = mutation - n=Amino-C6(or C2)-deoxythymine
  variation 35: note = mutation - n=Amino-C6(or C2)-deoxythymine
  source 1..50: mol_type = other DNA
tacantaagaggaaccaatttccgctgatagaatncccacaataagtctt

SEQ ID NO: 9 - DNA, 22 bp, synthetic construct
  misc_feature 1..22: note = Oligonucleotide
  source 1..22: mol_type = other DNA
gcctcacaatgttaatcttagc

SEQ ID NO: 10 - DNA, 18 bp, synthetic construct
  misc_feature 1..18: note = Oligonucleotide
  source 1..18: mol_type = other DNA
gattgtctcccatgaccg

SEQ ID NO: 11 - DNA, 42 bp, synthetic construct
  misc_feature 1..42: note = Oligonucleotide
  source 1..42: mol_type = other DNA
cctctatgcctcctaagtgccaatcgagaatatcctcctgaa

SEQ ID NO: 12 - DNA, 47 bp, synthetic construct
  misc_feature 1..47: note = Oligonucleotide
  source 1..47: mol_type = other DNA
gattacaacaaaaactgtggacgagctgatcgtaacttaaaaccagt

SEQ ID NO: 13 - DNA, 15 bp, synthetic construct
  misc_feature 1..15: note = Oligonucleotide
  source 1..15: mol_type = other DNA
ggtacgaactcgggc

SEQ ID NO: 14 - DNA, 20 bp, synthetic construct
  misc_feature 1..20: note = Oligonucleotide
  source 1..20: mol_type = other DNA
tgtgcacaaatctccttagt

SEQ ID NO: 15 - DNA, 42 bp, synthetic construct
  misc_feature 1..42: note = Oligonucleotide
  variation 5: note = mutation - n=Amino-C6(or C2)-deoxythymine
  variation 36: note = mutation - n=Amino-C6(or C2)-deoxythymine
  source 1..42: mol_type = other DNA
cctcnatgcctcctaagtgccaatcgagaatatccncctgaa

SEQ ID NO: 16 - DNA, 47 bp, synthetic construct
  misc_feature 1..47: note = Oligonucleotide
  variation 4: note = mutation - n=Amino-C6(or C2)-deoxythymine
  variation 37: note = mutation - n=Amino-C6(or C2)-deoxythymine
  source 1..47: mol_type = other DNA
gatnacaacaaaaactgtggacgagctgatcgtaacntaaaaccagt

SEQ ID NO: 17 - DNA, 22 bp, synthetic construct
  misc_feature 1..22: note = Oligonucleotide
  source 1..22: mol_type = other DNA
attacactataccatgaccctt

SEQ ID NO: 18 - DNA, 21 bp, synthetic construct
  misc_feature 1..21: note = Oligonucleotide
  source 1..21: mol_type = other DNA
cactgcctatgattaaagact

SEQ ID NO: 19 - DNA, 19 bp, synthetic construct
  misc_feature 1..19: note = probe
  source 1..19: mol_type = other DNA
cctcagataaacatctaac

SEQ ID NO: 20 - DNA, 21 bp, synthetic construct
  misc_feature 1..21: note = probe
  source 1..21: mol_type = other DNA
ggcctcagataaacatctaac

SEQ ID NO: 21 - DNA, 26 bp, synthetic construct
  misc_feature 1..26: note = probe
  source 1..26: mol_type = other DNA
tgtttggcctcagataaacatctaac

SEQ ID NO: 22 - DNA, 40 bp, synthetic construct
  misc_feature 1..40: note = probe
  source 1..40: mol_type = other DNA
ggctatcaaaataatgtttggcctcagataaacatctaac

SEQ ID NO: 23 - DNA, 19 bp, synthetic construct
  misc_feature 1..19: note = probe
  source 1..19: mol_type = other DNA
cggaaattggttcctctta